European Patent Application EP 4 755 451 A2, published June 10, 2026. Title: New treatment of SMA. Applicant: F. Hoffmann-La Roche AG. The sequence listing filed with the application follows.

SEQUENCE LISTING (9 sequences)

SEQ ID NO: 1 - DNA, 17 bp, Homo sapiens
  source 1..17: mol_type = other DNA
cccccaaggtgctgcta

SEQ ID NO: 2 - DNA, 21 bp, Homo sapiens
  source 1..21: mol_type = other DNA
tgaactggaagcaaaggagaa

SEQ ID NO: 3 - DNA, 20 bp, Homo sapiens
  source 1..20: mol_type = other DNA
ctttcttctgcaggaccagg

SEQ ID NO: 4 - DNA, 20 bp, Homo sapiens
  source 1..20: mol_type = other DNA
gaaggtgaaggtcggagtca

SEQ ID NO: 5 - DNA, 24 bp, Homo sapiens
  source 1..24: mol_type = other DNA
aaccatgtagttgaggtcaatgaa

SEQ ID NO: 6 - skipped

SEQ ID NO: 7 - DNA, 17 bp, Homo sapiens
  source 1..17: mol_type = other DNA
cccccaaggtgctgcta

SEQ ID NO: 8 - DNA, 21 bp, Homo sapiens
  source 1..21: mol_type = other DNA
tgaactggaagcaaaggacac

SEQ ID NO: 9 - DNA, 20 bp, Homo sapiens
  source 1..20: mol_type = other DNA
cttccttctgcagggccagg